European Patent Application EP 4 438 733 A2, published October 2, 2024. Title: ANTI-FUNGAL POLYPEPTIDES. Applicant: Biotalys NV. Application EP. The sequence listing filed with the application follows.

SEQUENCE LISTING (161 sequences)

SEQ ID NO: 1 - protein, 119 aa, synthetic construct
  REGION 1..119: note = 10G11Q
QVQLVESGGGLVQAGGSLRLSCAASRSIFSINAMDWYRQAPGKQREWVAGITRGGTTKYADSVKGRFTISRDNAKKKVYLQMNSLKPEDTAVYYCNVLRGEQPWTRDYWGQGTQVTVSS

SEQ ID NO: 2 - protein, 119 aa, synthetic construct
  REGION 1..119: note = 10G11
DVQLVESGGGLVQAGGSLRLSCAASRSIFSINAMDWYRQAPGKQREWVAGITRGGTTKYADSVKGRFTISRDNAKKKVYLQMNSLKPEDTAVYYCNVLRGEQPWTRDYWGQGTQVTVSS

SEQ ID NO: 3 - protein, 117 aa, synthetic construct
  REGION 1..117: note = 10E11Q
QVQLQESGGGLVQAGGSLRLSCAASGTIFRPTAMGWYRQAPGKERELVATITTGGSTKYADSVKGRFTISRGNAKNTVYLQMSSLKPEDTAVYYCNAQWGVRTRDYWGQGTQVTVSS

SEQ ID NO: 4 - protein, 117 aa, synthetic construct
  REGION 1..117: note = 10E11
DVQLQESGGGLVQAGGSLRLSCAASGTIFRPTAMGWYRQAPGKERELVATITTGGSTKYADSVKGRFTISRGNAKNTVYLQMSSLKPEDTAVYYCNAQWGVRTRDYWGQGTQVTVSS

SEQ ID NO: 5 - protein, 126 aa, synthetic construct
  REGION 1..126: note = 12C03Q
QVQLQESGGGLVQAGDSLRLSCAASISDRAFSRHVMGWFRQPPGKEREFVAAIGWTGRRTYYADSVKGRFTISRDNAMNTVYLQMNSLKPEDTAVYYCAASHFYSVSFEINDYDYWGQGTQVTVSS

SEQ ID NO: 6 - protein, 126 aa, synthetic construct
  REGION 1..126: note = 12C03
DVQLQESGGGLVQAGDSLRLSCAASISDRAFSRHVMGWFRQPPGKEREFVAAIGWTGRRTYYADSVKGRFTISRDNAMNTVYLQMNSLKPEDTAVYYCAASHFYSVSFEINDYDYWGQGTQVTVSS

SEQ ID NO: 7 - protein, 119 aa, synthetic construct
  REGION 1..119: note = Mutant 1
DVQLVESGGGLVQAGGSLRLSCAASASIFSINAMDWYRQAPGKQREWVAGITRGGTTKYADSVKGRFTISRDNAKKKVYLQMNSLKPEDTAVYYCNVLRGEQPWTRDYWGQGTQVTVSS

SEQ ID NO: 8 - protein, 119 aa, synthetic construct
  REGION 1..119: note = Mutant 2
DVQLVESGGGLVQAGGSLRLSCAASRSIFSINAMDWYRQAPGKQREWVAGITAGGTTAYADSVKGRFTISRDNAKKKVYLQMNSLKPEDTAVYYCNVLRGEQPWTRDYWGQGTQVTVSS

SEQ ID NO: 9 - protein, 119 aa, synthetic construct
  REGION 1..119: note = Mutant 3
DVQLVESGGGLVQAGGSLRLSCAASRSIFSINAMDWYRQAPGKQREWVAGITRGGTTKYADSVKGRFTISRDNAKKKVYLQMNSLKPEDTAVYYCNVLAGEQPWTADYWGQGTQVTVSS

SEQ ID NO: 10 - protein, 119 aa, synthetic construct
  REGION 1..119: note = Mutant 4
DVQLVESGGGLVQAGGSLRLSCAASASIFSINAMDWYRQAPGKQREWVAGITAGGTTAYADSVKGRFTISRDNAKKKVYLQMNSLKPEDTAVYYCNVLAGEQPWTADYWGQGTQVTVSS

SEQ ID NO: 11 - protein, 119 aa, synthetic construct
  REGION 1..119: note = Mutant 5
DVQLVESGGGLVQAGGSLRLSCAASASIFSINAMDWYRQAPGKQREWVAGITAGGTTAYADSVKGRFTISRDNAKNTVYLQMNSLKPEDTAVYYCNVLAGEQPWTADYWGQGTQVTVSS

SEQ ID NO: 12 - protein, 119 aa, synthetic construct
  REGION 1..119: note = Mutant 6
DVQLVESGGGLVQAGGSLRLSCAASRHHFHINAMDWYRQAPGKQREWVAGITRGGTTKYADSVKGRFTISRDNAKKKVYLQMNSLKPEDTAVYYCNVLRGEQPWTRDYWGQGTQVTVSS

SEQ ID NO: 13 - protein, 119 aa, synthetic construct
  REGION 1..119: note = Mutant 7
DVQLVESGGGLVQAGGSLRLSCAASRSIFSINAMDWYRQAPGKQREWVAGITRGGTTKYADSVKGRFTISRDNAKKKVYLQMNSLKPEDTAVYYCNVLRGEQPHHRDYWGQGTQVTVSS

SEQ ID NO: 14 - protein, 119 aa, synthetic construct
  REGION 1..119: note = Mutant 8
DVQLVESGGGLVQAGGSLRLSCAASRHHFHINAMDWYRQAPGKQREWVAGITRGGTTKYADSVKGRFTISRDNAKKKVYLQMNSLKPEDTAVYYCNVLRGEQPHHRDYWGQGTQVTVSS

SEQ ID NO: 15 - protein, 119 aa, synthetic construct
  REGION 1..119: note = Mutant 9
DVQLVESGGGLVQAGGSLRLSCAASRKKFKINAMDWYRQAPGKQREWVAGITRGGTTKYADSVKGRFTISRDNAKKKVYLQMNSLKPEDTAVYYCNVLRGEQPWTRDYWGQGTQVTVSS

SEQ ID NO: 16 - protein, 119 aa, synthetic construct
  REGION 1..119: note = Mutant 10
DVQLVESGGGLVQAGGSLRLSCAASRSIFSINAMDWYRQAPGKQREWVAGITRGGTTKYADSVKGRFTISRDNAKKKVYLQMNSLKPEDTAVYYCNVLRGEQPKKRDYWGQGTQVTVSS

SEQ ID NO: 17 - protein, 119 aa, synthetic construct
  REGION 1..119: note = Mutant 11
DVQLVESGGGLVQAGGSLRLSCAASRKKFKINAMDWYRQAPGKQREWVAGITRGGTTKYADSVKGRFTISRDNAKKKVYLQMNSLKPEDTAVYYCNVLRGEQPKKRDYWGQGTQVTVSS

SEQ ID NO: 18 - protein, 119 aa, synthetic construct
  REGION 1..119: note = Single ALA mutant 1
DVQLVESGGGLVQAGGSLRLSCAASGSIFSINAMDWYRQAPGKQREWVAGITRGGTTKYADSVKGRFTISRDNAKKKVYLQMNSLKPEDTAVYYCNVLRGEQPWTRDYWGQGTQVTVSS

SEQ ID NO: 19 - protein, 119 aa, synthetic construct
  REGION 1..119: note = Single ALA mutant 2
DVQLVESGGGLVQAGGSLRLSCAASRAIFSINAMDWYRQAPGKQREWVAGITRGGTTKYADSVKGRFTISRDNAKKKVYLQMNSLKPEDTAVYYCNVLRGEQPWTRDYWGQGTQVTVSS

SEQ ID NO: 20 - protein, 119 aa, synthetic construct
  REGION 1..119: note = Single ALA mutant 3
DVQLVESGGGLVQAGGSLRLSCAASRSAFSINAMDWYRQAPGKQREWVAGITRGGTTKYADSVKGRFTISRDNAKKKVYLQMNSLKPEDTAVYYCNVLRGEQPWTRDYWGQGTQVTVSS

SEQ ID NO: 21 - protein, 119 aa, synthetic construct
  REGION 1..119: note = Single ALA mutant 4
DVQLVESGGGLVQAGGSLRLSCAASRSIASINAMDWYRQAPGKQREWVAGITRGGTTKYADSVKGRFTISRDNAKKKVYLQMNSLKPEDTAVYYCNVLRGEQPWTRDYWGQGTQVTVSS

SEQ ID NO: 22 - protein, 119 aa, synthetic construct
  REGION 1..119: note = Single ALA mutant 5
DVQLVESGGGLVQAGGSLRLSCAASRSIFAINAMDWYRQAPGKQREWVAGITRGGTTKYADSVKGRFTISRDNAKKKVYLQMNSLKPEDTAVYYCNVLRGEQPWTRDYWGQGTQVTVSS

SEQ ID NO: 23 - protein, 119 aa, synthetic construct
  REGION 1..119: note = Single ALA mutant 6
DVQLVESGGGLVQAGGSLRLSCAASRSIFSANAMDWYRQAPGKQREWVAGITRGGTTKYADSVKGRFTISRDNAKKKVYLQMNSLKPEDTAVYYCNVLRGEQPWTRDYWGQGTQVTVSS

SEQ ID NO: 24 - protein, 119 aa, synthetic construct
  REGION 1..119: note = Single ALA mutant 7
DVQLVESGGGLVQAGGSLRLSCAASRSIFSIAAMDWYRQAPGKQREWVAGITRGGTTKYADSVKGRFTISRDNAKKKVYLQMNSLKPEDTAVYYCNVLRGEQPWTRDYWGQGTQVTVSS

SEQ ID NO: 25 - protein, 119 aa, synthetic construct
  REGION 1..119: note = Single ALA mutant 8
DVQLVESGGGLVQAGGSLRLSCAASRSIFSINAADWYRQAPGKQREWVAGITRGGTTKYADSVKGRFTISRDNAKKKVYLQMNSLKPEDTAVYYCNVLRGEQPWTRDYWGQGTQVTVSS

SEQ ID NO: 26 - protein, 119 aa, synthetic construct
  REGION 1..119: note = Single ALA mutant 9
DVQLVESGGGLVQAGGSLRLSCAASRSIFSINAMAWYRQAPGKQREWVAGITRGGTTKYADSVKGRFTISRDNAKKKVYLQMNSLKPEDTAVYYCNVLRGEQPWTRDYWGQGTQVTVSS

SEQ ID NO: 27 - protein, 119 aa, synthetic construct
  REGION 1..119: note = Single ALA mutant 10
DVQLVESGGGLVQAGGSLRLSCAASRSIFSINAMGWYRQAPGKQREWVAGITRGGTTKYADSVKGRFTISRDNAKKKVYLQMNSLKPEDTAVYYCNVLRGEQPWTRDYWGQGTQVTVSS

SEQ ID NO: 28 - protein, 119 aa, synthetic construct
  REGION 1..119: note = Single ALA mutant 11
DVQLVESGGGLVQAGGSLRLSCAASRSIFSINAMDWYRQAPGKQREWVAAITRGGTTKYADSVKGRFTISRDNAKKKVYLQMNSLKPEDTAVYYCNVLRGEQPWTRDYWGQGTQVTVSS

SEQ ID NO: 29 - protein, 119 aa, synthetic construct
  REGION 1..119: note = Single ALA mutant 12
DVQLVESGGGLVQAGGSLRLSCAASRSIFSINAMDWYRQAPGKQREWVAGATRGGTTKYADSVKGRFTISRDNAKKKVYLQMNSLKPEDTAVYYCNVLRGEQPWTRDYWGQGTQVTVSS

SEQ ID NO: 30 - protein, 119 aa, synthetic construct
  REGION 1..119: note = Single ALA mutant 13
DVQLVESGGGLVQAGGSLRLSCAASRSIFSINAMDWYRQAPGKQREWVAGIARGGTTKYADSVKGRFTISRDNAKKKVYLQMNSLKPEDTAVYYCNVLRGEQPWTRDYWGQGTQVTVSS

SEQ ID NO: 31 - protein, 119 aa, synthetic construct
  REGION 1..119: note = Single ALA mutant 14
DVQLVESGGGLVQAGGSLRLSCAASRSIFSINAMDWYRQAPGKQREWVAGITAGGTTKYADSVKGRFTISRDNAKKKVYLQMNSLKPEDTAVYYCNVLRGEQPWTRDYWGQGTQVTVSS

SEQ ID NO: 32 - protein, 119 aa, synthetic construct
  REGION 1..119: note = Single ALA mutant 15
DVQLVESGGGLVQAGGSLRLSCAASRSIFSINAMDWYRQAPGKQREWVAGITSGGTTKYADSVKGRFTISRDNAKKKVYLQMNSLKPEDTAVYYCNVLRGEQPWTRDYWGQGTQVTVSS

SEQ ID NO: 33 - protein, 119 aa, synthetic construct
  REGION 1..119: note = Single ALA mutant 16
DVQLVESGGGLVQAGGSLRLSCAASRSIFSINAMDWYRQAPGKQREWVAGITRAGTTKYADSVKGRFTISRDNAKKKVYLQMNSLKPEDTAVYYCNVLRGEQPWTRDYWGQGTQVTVSS

SEQ ID NO: 34 - protein, 119 aa, synthetic construct
  REGION 1..119: note = Single ALA mutant 17
DVQLVESGGGLVQAGGSLRLSCAASRSIFSINAMDWYRQAPGKQREWVAGITRGATTKYADSVKGRFTISRDNAKKKVYLQMNSLKPEDTAVYYCNVLRGEQPWTRDYWGQGTQVTVSS

SEQ ID NO: 35 - protein, 119 aa, synthetic construct
  REGION 1..119: note = Single ALA mutant 18
DVQLVESGGGLVQAGGSLRLSCAASRSIFSINAMDWYRQAPGKQREWVAGITRGGATKYADSVKGRFTISRDNAKKKVYLQMNSLKPEDTAVYYCNVLRGEQPWTRDYWGQGTQVTVSS

SEQ ID NO: 36 - protein, 119 aa, synthetic construct
  REGION 1..119: note = Single ALA mutant 19
DVQLVESGGGLVQAGGSLRLSCAASRSIFSINAMDWYRQAPGKQREWVAGITRGGSTKYADSVKGRFTISRDNAKKKVYLQMNSLKPEDTAVYYCNVLRGEQPWTRDYWGQGTQVTVSS

SEQ ID NO: 37 - protein, 119 aa, synthetic construct
  REGION 1..119: note = Single ALA mutant 20
DVQLVESGGGLVQAGGSLRLSCAASRSIFSINAMDWYRQAPGKQREWVAGITRGGTAKYADSVKGRFTISRDNAKKKVYLQMNSLKPEDTAVYYCNVLRGEQPWTRDYWGQGTQVTVSS

SEQ ID NO: 38 - protein, 119 aa, synthetic construct
  REGION 1..119: note = Single ALA mutant 21
DVQLVESGGGLVQAGGSLRLSCAASRSIFSINAMDWYRQAPGKQREWVAGITRGGTTAYADSVKGRFTISRDNAKKKVYLQMNSLKPEDTAVYYCNVLRGEQPWTRDYWGQGTQVTVSS

SEQ ID NO: 39 - protein, 119 aa, synthetic construct
  REGION 1..119: note = Single ALA mutant 22
DVQLVESGGGLVQAGGSLRLSCAASRSIFSINAMDWYRQAPGKQREWVAGITRGGTTNYADSVKGRFTISRDNAKKKVYLQMNSLKPEDTAVYYCNVLRGEQPWTRDYWGQGTQVTVSS

SEQ ID NO: 40 - protein, 119 aa, synthetic construct
  REGION 1..119: note = Single ALA mutant 23
DVQLVESGGGLVQAGGSLRLSCAASRSIFSINAMDWYRQAPGKQREWVAGITRGGTTKYADSVKGRFTISRDNAKKKVYLQMNSLKPEDTAVYYCNALRGEQPWTRDYWGQGTQVTVSS

SEQ ID NO: 41 - protein, 119 aa, synthetic construct
  REGION 1..119: note = Single ALA mutant 24
DVQLVESGGGLVQAGGSLRLSCAASRSIFSINAMDWYRQAPGKQREWVAGITRGGTTKYADSVKGRFTISRDNAKKKVYLQMNSLKPEDTAVYYCNVARGEQPWTRDYWGQGTQVTVSS

SEQ ID NO: 42 - protein, 119 aa, synthetic construct
  REGION 1..119: note = Single ALA mutant 25
DVQLVESGGGLVQAGGSLRLSCAASRSIFSINAMDWYRQAPGKQREWVAGITRGGTTKYADSVKGRFTISRDNAKKKVYLQMNSLKPEDTAVYYCNVLAGEQPWTRDYWGQGTQVTVSS

SEQ ID NO: 43 - protein, 119 aa, synthetic construct
  REGION 1..119: note = Single ALA mutant 26
DVQLVESGGGLVQAGGSLRLSCAASRSIFSINAMDWYRQAPGKQREWVAGITRGGTTKYADSVKGRFTISRDNAKKKVYLQMNSLKPEDTAVYYCNVLRAEQPWTRDYWGQGTQVTVSS

SEQ ID NO: 44 - protein, 119 aa, synthetic construct
  REGION 1..119: note = Single ALA mutant 27
DVQLVESGGGLVQAGGSLRLSCAASRSIFSINAMDWYRQAPGKQREWVAGITRGGTTKYADSVKGRFTISRDNAKKKVYLQMNSLKPEDTAVYYCNVLRGAQPWTRDYWGQGTQVTVSS

SEQ ID NO: 45 - protein, 119 aa, synthetic construct
  REGION 1..119: note = Single ALA mutant 28
DVQLVESGGGLVQAGGSLRLSCAASRSIFSINAMDWYRQAPGKQREWVAGITRGGTTKYADSVKGRFTISRDNAKKKVYLQMNSLKPEDTAVYYCNVLRGEAPWTRDYWGQGTQVTVSS

SEQ ID NO: 46 - protein, 119 aa, synthetic construct
  REGION 1..119: note = Single ALA mutant 29
DVQLVESGGGLVQAGGSLRLSCAASRSIFSINAMDWYRQAPGKQREWVAGITRGGTTKYADSVKGRFTISRDNAKKKVYLQMNSLKPEDTAVYYCNVLRGEQAWTRDYWGQGTQVTVSS

SEQ ID NO: 47 - protein, 119 aa, synthetic construct
  REGION 1..119: note = Single ALA mutant 30
DVQLVESGGGLVQAGGSLRLSCAASRSIFSINAMDWYRQAPGKQREWVAGITRGGTTKYADSVKGRFTISRDNAKKKVYLQMNSLKPEDTAVYYCNVLRGEQPATRDYWGQGTQVTVSS

SEQ ID NO: 48 - protein, 119 aa, synthetic construct
  REGION 1..119: note = Single ALA mutant 31
DVQLVESGGGLVQAGGSLRLSCAASRSIFSINAMDWYRQAPGKQREWVAGITRGGTTKYADSVKGRFTISRDNAKKKVYLQMNSLKPEDTAVYYCNVLRGEQPWARDYWGQGTQVTVSS

SEQ ID NO: 49 - protein, 119 aa, synthetic construct
  REGION 1..119: note = Single ALA mutant 32
DVQLVESGGGLVQAGGSLRLSCAASRSIFSINAMDWYRQAPGKQREWVAGITRGGTTKYADSVKGRFTISRDNAKKKVYLQMNSLKPEDTAVYYCNVLRGEQPWTADYWGQGTQVTVSS

SEQ ID NO: 50 - protein, 119 aa, synthetic construct
  REGION 1..119: note = Single ALA mutant 33
DVQLVESGGGLVQAGGSLRLSCAASRSIFSINAMDWYRQAPGKQREWVAGITRGGTTKYADSVKGRFTISRDNAKKKVYLQMNSLKPEDTAVYYCNVLRGEQPWTRAYWGQGTQVTVSS

SEQ ID NO: 51 - protein, 119 aa, synthetic construct
  REGION 1..119: note = Single ALA mutant 34
DVQLVESGGGLVQAGGSLRLSCAASRSIFSINAMDWYRQAPGKQREWVAGITRGGTTKYADSVKGRFTISRDNAKKKVYLQMNSLKPEDTAVYYCNVLRGEQPWTRDAWGQGTQVTVSS

SEQ ID NO: 52 - protein, 10 aa, synthetic construct
  REGION 1..10: note = CDR1-10G11 (and CDR1-10G11Q)
RSIFSINAMD

SEQ ID NO: 53 - protein, 10 aa, synthetic construct
  REGION 1..10: note = CDR1-10E11 (and CDR1-10E11Q)
GTIFRPTAMG

SEQ ID NO: 54 - protein, 10 aa, synthetic construct
  REGION 1..10: note = CDR1-12C03 (and CDR1-12C03Q)
ISDRAFSRHV

SEQ ID NO: 55 - protein, 10 aa, synthetic construct
  REGION 1..10: note = CDR1-Mutant 1
ASIFSINAMD

SEQ ID NO: 56 - protein, 10 aa, synthetic construct
  REGION 1..10: note = CDR1-Mutant 6 and 8
RHHFHINAMD

SEQ ID NO: 57 - protein, 10 aa, synthetic construct
  REGION 1..10: note = CDR1-Mutant 9 and 11
RKKFKINAMD

SEQ ID NO: 58 - protein, 10 aa, synthetic construct
  REGION 1..10: note = CDR1-Single ALA mutant 1
GSIFSINAMD

SEQ ID NO: 59 - protein, 10 aa, synthetic construct
  REGION 1..10: note = CDR1-Single ALA mutant 2
RAIFSINAMD

SEQ ID NO: 60 - protein, 10 aa, synthetic construct
  REGION 1..10: note = CDR1-Single ALA mutant 3
RSAFSINAMD

SEQ ID NO: 61 - protein, 10 aa, synthetic construct
  REGION 1..10: note = CDR1-Single ALA mutant 4
RSIASINAMD

SEQ ID NO: 62 - protein, 10 aa, synthetic construct
  REGION 1..10: note = CDR1-Single ALA mutant 5
RSIFAINAMD

SEQ ID NO: 63 - protein, 10 aa, synthetic construct
  REGION 1..10: note = CDR1-Single ALA mutant 6
RSIFSANAMD

SEQ ID NO: 64 - protein, 10 aa, synthetic construct
  REGION 1..10: note = CDR1-Single ALA mutant 7
RSIFSIAAMD

SEQ ID NO: 65 - protein, 10 aa, synthetic construct
  REGION 1..10: note = CDR1-Single ALA mutant 8
RSIFSINAAD

SEQ ID NO: 66 - protein, 10 aa, synthetic construct
  REGION 1..10: note = CDR1-Single ALA mutant 9
RSIFSINAMA

SEQ ID NO: 67 - protein, 10 aa, synthetic construct
  REGION 1..10: note = CDR1-Single ALA mutant 10
RSIFSINAMG

SEQ ID NO: 68 - protein, 9 aa, synthetic construct
  REGION 1..9: note = CDR2-10G11 (and CDR2-10G11Q)
GITRGGTTK

SEQ ID NO: 69 - protein, 9 aa, synthetic construct
  REGION 1..9: note = CDR2-10E11 (and CDR2-10E11Q)
TITTGGSTK

SEQ ID NO: 70 - protein, 10 aa, synthetic construct
  REGION 1..10: note = CDR2-12C03 (and CDR2-12C03Q)
AIGWTGRRTY

SEQ ID NO: 71 - protein, 9 aa, synthetic construct
  REGION 1..9: note = CDR2-Mutant 2
GITAGGTTA

SEQ ID NO: 72 - protein, 9 aa, synthetic construct
  REGION 1..9: note = CDR2-Single ALA mutant 11
AITRGGTTK

SEQ ID NO: 73 - protein, 9 aa, synthetic construct
  REGION 1..9: note = CDR2-Single ALA mutant 12
GATRGGTTK

SEQ ID NO: 74 - protein, 9 aa, synthetic construct
  REGION 1..9: note = CDR2-Single ALA mutant 13
GIARGGTTK

SEQ ID NO: 75 - protein, 9 aa, synthetic construct
  REGION 1..9: note = CDR2-Single ALA mutant 14
GITAGGTTK

SEQ ID NO: 76 - protein, 9 aa, synthetic construct
  REGION 1..9: note = CDR2-Single ALA mutant 15
GITSGGTTK

SEQ ID NO: 77 - protein, 9 aa, synthetic construct
  REGION 1..9: note = CDR2-Single ALA mutant 16
GITRAGTTK

SEQ ID NO: 78 - protein, 9 aa, synthetic construct
  REGION 1..9: note = CDR2-Single ALA mutant 17
GITRGATTK

SEQ ID NO: 79 - protein, 9 aa, synthetic construct
  REGION 1..9: note = CDR2-Single ALA mutant 18
GITRGGATK

SEQ ID NO: 80 - protein, 9 aa, synthetic construct
  REGION 1..9: note = CDR2-Single ALA mutant 19
GITRGGSTK

SEQ ID NO: 81 - protein, 9 aa, synthetic construct
  REGION 1..9: note = CDR2-Single ALA mutant 20
GITRGGTAK

SEQ ID NO: 82 - protein, 9 aa, synthetic construct
  REGION 1..9: note = CDR2-Single ALA mutant 21
GITRGGTTA

SEQ ID NO: 83 - protein, 9 aa, synthetic construct
  REGION 1..9: note = CDR2-Single ALA mutant 22
GITRGGTTN

SEQ ID NO: 84 - protein, 11 aa, synthetic construct
  REGION 1..11: note = CDR3-10G11 (and CDR3-10G11Q)
LRGEQPWTRDY

SEQ ID NO: 85 - protein, 9 aa, synthetic construct
  REGION 1..9: note = CDR3-10E11 (and CDR3-10E11Q)
QWGVRTRDY

SEQ ID NO: 86 - protein, 15 aa, synthetic construct
  REGION 1..15: note = CDR3-12C03 (and CDR3-12C03Q)
SHFYSVSFEINDYDY

SEQ ID NO: 87 - protein, 11 aa, synthetic construct
  REGION 1..11: note = CDR3-Mutant 3
LAGEQPWTADY

SEQ ID NO: 88 - protein, 11 aa, synthetic construct
  REGION 1..11: note = CDR3-Mutant 7
LRGEQPHHRDY

SEQ ID NO: 89 - protein, 11 aa, synthetic construct
  REGION 1..11: note = CDR3-Mutant 10
LRGEQPKKRDY

SEQ ID NO: 90 - protein, 11 aa, synthetic construct
  REGION 1..11: note = CDR3-Single ALA mutant 24
ARGEQPWTRDY

SEQ ID NO: 91 - protein, 11 aa, synthetic construct
  REGION 1..11: note = CDR3-Single ALA mutant 25
LAGEQPWTRDY

SEQ ID NO: 92 - protein, 11 aa, synthetic construct
  REGION 1..11: note = CDR3-Single ALA mutant 26
LRAEQPWTRDY

SEQ ID NO: 93 - protein, 11 aa, synthetic construct
  REGION 1..11: note = CDR3-Single ALA mutant 27
LRGAQPWTRDY

SEQ ID NO: 94 - protein, 11 aa, synthetic construct
  REGION 1..11: note = CDR3-Single ALA mutant 28
LRGEAPWTRDY

SEQ ID NO: 95 - protein, 11 aa, synthetic construct
  REGION 1..11: note = CDR3-Single ALA mutant 29
LRGEQAWTRDY

SEQ ID NO: 96 - protein, 11 aa, synthetic construct
  REGION 1..11: note = CDR3-Single ALA mutant 30
LRGEQPATRDY

SEQ ID NO: 97 - protein, 11 aa, synthetic construct
  REGION 1..11: note = CDR3-Single ALA mutant 31
LRGEQPWARDY

SEQ ID NO: 98 - protein, 11 aa, synthetic construct
  REGION 1..11: note = CDR3-Single ALA mutant 32
LRGEQPWTADY

SEQ ID NO: 99 - protein, 11 aa, synthetic construct
  REGION 1..11: note = CDR3-Single ALA mutant 33
LRGEQPWTRAY

SEQ ID NO: 100 - protein, 11 aa, synthetic construct
  REGION 1..11: note = CDR3-Single ALA mutant 34
LRGEQPWTRDA

SEQ ID NO: 101 - protein, 119 aa, synthetic construct
  REGION 1..119: note = 10G11 General Formula A
  SITE 1: note = misc_feature - X is D or Q
  REGION 26..28: note = misc_feature - X is G, A, V, L, I, M, P, F, W, S, T, N, Q, Y, C, K, R, H, D or E
  SITE 30: note = misc_feature - X is G, A, V, L, I, M, P, F, W, S, T, N, Q, Y, C, K, R, H, D or E
  SITE 53: note = misc_feature - X is G, A, V, L, I, M, P, F, W, S, T, N, Q, Y, C, K, R, H, D or E
  SITE 58: note = misc_feature - X is G, A, V, L, I, M, P, F, W, S, T, N, Q, Y, C, K, R, H, D or E
  SITE 99: note = misc_feature - X is G, A, V, L, I, M, P, F, W, S, T, N, Q, Y, C, K, R, H, D or E
  REGION 104..106: note = misc_feature - X is G, A, V, L, I, M, P, F, W, S, T, N, Q, Y, C, K, R, H, D or E
XVQLVESGGGLVQAGGSLRLSCAASXXXFXINAMDWYRQAPGKQREWVAGITXGGTTXYADSVKGRFTISRDNAKKKVYLQMNSLKPEDTAVYYCNVLXGEQPXXXDYWGQGTQVTVSS

SEQ ID NO: 102 - protein, 119 aa, synthetic construct; identical to SEQ ID NO: 101
  REGION 1..119: note = 10G11 General Formula B
  SITE 1: note = misc_feature - X is D or Q
  REGION 26..28: note = misc_feature - X is G, A, V, L, I, M, P, F, W, S, T, N, Q, Y, C, K, R or H
  SITE 30: note = misc_feature - X is G, A, V, L, I, M, P, F, W, S, T, N, Q, Y, C, K, R or H
  SITE 53: note = misc_feature - X is G, A, V, L, I, M, P, F, W, S, T, N, Q, Y, C, K, R or H
  SITE 58: note = misc_feature - X is G, A, V, L, I, M, P, F, W, S, T, N, Q, Y, C, K, R or H
  SITE 99: note = misc_feature - X is G, A, V, L, I, M, P, F, W, S, T, N, Q, Y, C, K, R or H
  REGION 104..106: note = misc_feature - X is G, A, V, L, I, M, P, F, W, S, T, N, Q, Y, C, K, R or H

SEQ ID NO: 103 - protein, 119 aa, synthetic construct; identical to SEQ ID NO: 101
  REGION 1..119: note = 10G11 General Formula C
  SITE 1: note = misc_feature - X is D or Q
  SITE 26: note = misc_feature - X is G, A, V, M, L, I, K, R or H
  REGION 27..28: note = misc_feature - X is G, A, V, L, I, M, P, F, W, S, T, N, Q, Y, C, K, R or H
  REGION 27..28: note = misc_feature - X is G, A, V, L, I, M, P, F, W, S, T, N, Q, Y, C, K, R or H
  SITE 30: note = misc_feature - X is G, A, V, L, I, M, P, F, W, S, T, N, Q, Y, C, K, R or H
  SITE 53: note = misc_feature - X is G, A, V, M, L, I, K, R, H
  SITE 58: note = misc_feature - X is G, A, V, M, L, I, K, R, H
  SITE 99: note = misc_feature - X is G, A, V, M, L, I, K, R, or H
  REGION 104..105: note = misc_feature - X is G, A, V, L, I, M, P, F, W, S, T, N, Q, Y, C, K, R or H
  SITE 106: note = misc_feature - X is G, A, V, M, L, I, K, R, or H

SEQ ID NO: 104 - protein, 119 aa, synthetic construct; identical to SEQ ID NO: 101
  REGION 1..119: note = 10G11 General Formula D
  SITE 1: note = misc_feature - X is D or Q
  SITE 26: note = misc_feature - X is A, K, R or H
  REGION 27..28: note = misc_feature - X is any naturally occurring amino acid, except for E or D
  REGION 27..28: note = misc_feature - X is any naturally occurring amino acid, except for E or D
  REGION 27..28: note = misc_feature - X is any naturally occurring amino acid, except for E or D
  SITE 30: note = misc_feature - X is G, A, V, L, I, M, P, F, W, S, T, N, Q, Y, C, K, R or H
  SITE 53: note = misc_feature - X is A, R, K or H
  SITE 53: note = misc_feature - X is A, R, K or H
  SITE 58: note = misc_feature - X is A, R, K or H
  SITE 99: note = misc_feature - X is A, R, K or H
  REGION 104..105: note = misc_feature - X is G, A, V, L, I, M, P, F, W, S, T, N, Q, Y, C, K, R or H
  SITE 106: note = misc_feature - X is A, R, K or H

SEQ ID NO: 105 - protein, 119 aa, synthetic construct; identical to SEQ ID NO: 101
  REGION 1..119: note = 10G11 General Formula E
  SITE 1: note = misc_feature - X is D or Q
  SITE 26: note = misc_feature - X is A, R, K, H
  SITE 27: note = misc_feature - X is S, T, C, P, N, Q, R or H
  SITE 28: note = misc_feature - X is I, G, A, V, M, L, K, R, or H
  SITE 30: note = misc_feature - X is S, T, C, P, N, Q, K, R or H
  SITE 53: note = misc_feature - X is A, K, R or H
  SITE 58: note = misc_feature - X is A, K, R or H
  SITE 58: note = misc_feature - X is A, K, R or H
  SITE 99: note = misc_feature - X is A, K, R or H
  SITE 104: note = misc_feature - X is W, F, Y, K, R or H
  SITE 105: note = misc_feature - X is S, T, C, P, N, Q, K, R or H
  SITE 106: note = misc_feature - X is A, K, R or H

SEQ ID NO: 106 - protein, 119 aa, synthetic construct; identical to SEQ ID NO: 101
  REGION 1..119: note = 10G11 General Formula F
  SITE 1: note = misc_feature - X is D or Q
  SITE 26: note = misc_feature - X is A, K, R, H
  SITE 27: note = misc_feature - X is S, K, R, H
  SITE 28: note = misc_feature - X is I, K, R, H
  SITE 30: note = misc_feature - X is S, K, R, H
  SITE 53: note = misc_feature - X is A, K, R, H
  SITE 58: note = misc_feature - X is A, K, R, H
  SITE 99: note = misc_feature - X is A, K, R, H
  SITE 104: note = misc_feature - X is W, K, R, H
  SITE 105: note = misc_feature - X is T, K, R, H
  SITE 106: note = misc_feature - X is A, K, R, H

SEQ ID NO: 107 - protein, 119 aa, synthetic construct; identical to SEQ ID NO: 101
  REGION 1..119: note = 10G11 General Formula G
  SITE 1: note = misc_feature - X is D or Q
  SITE 26: note = misc_feature - X is K, R, H
  SITE 27: note = misc_feature - X is S, K, R, H
  SITE 28: note = misc_feature - X is I, K, R, H
  SITE 30: note = misc_feature - X is S, K, R, H
  SITE 53: note = misc_feature - X is K, R, H
  SITE 58: note = misc_feature - X is K, R, H
  SITE 99: note = misc_feature - X is K, R, H
  SITE 104: note = misc_feature - X is W, K, R, H
  SITE 105: note = misc_feature - X is T, K, R, H
  SITE 106: note = misc_feature - X is A, K, R, H

SEQ ID NO: 108 - protein, 119 aa, synthetic construct
  REGION 1..119: note = 10G11 General Formula H
  SITE 1: note = misc_feature - X is D or Q
  REGION 27..28: note = misc_feature - X is any naturally occurring amino acid
  SITE 30: note = misc_feature - X is G, A, V, L, I, M, P, F, W, S, T, N, Q, Y, C, K, R, H, D, E
  REGION 104..105: note = misc_feature - X is G, A, V, L, I, M, P, F, W, S, T, N, Q, Y, C, K, R, H, D, E
XVQLVESGGGLVQAGGSLRLSCAASRXXFXINAMDWYRQAPGKQREWVAGITRGGTTKYADSVKGRFTISRDNAKKKVYLQMNSLKPEDTAVYYCNVLRGEQPXXRDYWGQGTQVTVSS

SEQ ID NO: 109 - protein, 119 aa, synthetic construct; identical to SEQ ID NO: 108
  REGION 1..119: note = 10G11 General Formula I
  SITE 1: note = misc_feature - X is D or Q
  REGION 27..28: note = misc_feature - X is G, A, V, L, I, M, P, F, W, S, T, N, Q, Y, C, K, R or H
  SITE 30: note = misc_feature - X is G, A, V, L, I, M, P, F, W, S, T, N, Q, Y, C, K, R or H
  REGION 104..105: note = misc_feature - X is G, A, V, L, I, M, P, F, W, S, T, N, Q, Y, C, K, R or H

SEQ ID NO: 110 - protein, 119 aa, synthetic construct; identical to SEQ ID NO: 108
  REGION 1..119: note = 10G11 General Formula J
  SITE 1: note = misc_feature - X is D or Q
  SITE 27: note = misc_feature - X is S, T, C, P, N, Q, K, R, H
  SITE 28: note = misc_feature - X is I, G, A, V, M, L, K, R, H
  SITE 28: note = misc_feature - X is I, G, A, V, M, L, K, R, H
  SITE 30: note = misc_feature - X is S, T, C, P, N, Q, K, R, H
  SITE 104: note = misc_feature - X is W, F, Y, K, R, H
  SITE 105: note = misc_feature - X is S, T, C, P, N, Q, K, R, H

SEQ ID NO: 111 - protein, 119 aa, synthetic construct; identical to SEQ ID NO: 108
  REGION 1..119: note = 10G11 General Formula K
  SITE 1: note = misc_feature - X is D or Q
  SITE 27: note = misc_feature - X is S, K, R, H
  SITE 28: note = misc_feature - X is I, K, R, H
  SITE 30: note = misc_feature - X is S, K, R, H
  SITE 104: note = misc_feature - X is W, K, R, H
  SITE 105: note = misc_feature - X is T, K, R, H

SEQ ID NO: 112 - protein, 10 aa, synthetic construct
  REGION 1..10: note = 10G11 General Formula CDR1 A
  REGION 1..3: note = misc_feature - X is G, A, V, L, I, M, P, F, W, S, T, N, Q, Y, C, K, R, H. D, E
  SITE 5: note = misc_feature - X is G, A, V, L, I, M, P, F, W, S, T, N, Q, Y, C, K, R, H. D, E
XXXFXINAMD

SEQ ID NO: 113 - protein, 10 aa, synthetic construct
  REGION 1..10: note = 10G11 General Formula CDR1 B
  REGION 1..3: note = misc_feature - X is G, A, V, L, I, M, P, F, W, S, T, N, Q, Y, C, K, R, H
  SITE 5: note = misc_feature - X is G, A, V, L, I, M, P, F, W, S, T, N, Q, Y, C, K, R, H
XXXFXINAMD

SEQ ID NO: 114 - protein, 10 aa, synthetic construct
  REGION 1..10: note = 10G11 General Formula CDR1 C
  SITE 1: note = misc_feature - X is G, A, V, M, L, I, K, R, H
  REGION 2..3: note = misc_feature - X is G, A, V, L, I, M, P, F, W, S, T, N, Q, Y, C, K, R or H
  SITE 5: note = misc_feature - X is G, A, V, L, I, M, P, F, W, S, T, N, Q, Y, C, K, R or H
XXXFXINAMD

SEQ ID NO: 115 - protein, 10 aa, synthetic construct
  REGION 1..10: note = 10G11 General Formula CDR1 D
  SITE 1: note = misc_feature - X is A, K, R, H
  REGION 2..3: note = misc_feature - X is G, A, V, L, I, M, P, F, W, S, T, N, Q, Y, C, K, R, H
  SITE 5: note = misc_feature - X is G, A, V, L, I, M, P, F, W, S, T, N, Q, Y, C, K, R, H
XXXFXINAMD

SEQ ID NO: 116 - protein, 10 aa, synthetic construct
  REGION 1..10: note = 10G11 General Formula CDR1 E
  SITE 1: note = misc_feature - X is A, K, R, H
  SITE 2: note = misc_feature - X is S, T, C, P, N, Q, K, R, H
  SITE 3: note = misc_feature - X is I, G, A, V, M, L, K, R, H
  SITE 5: note = misc_feature - X is S, T, C, P, N, Q, K, R, H
XXXFXINAMD

SEQ ID NO: 117 - protein, 10 aa, synthetic construct
  REGION 1..10: note = 10G11 General Formula CDR1 F
  SITE 1: note = misc_feature - X is A, K, R, H
  SITE 2: note = misc_feature - X is S, K, R, H
  SITE 3: note = misc_feature - X is I, K, R, H
  SITE 5: note = misc_feature - X is S, K, R, H
XXXFXINAMD

SEQ ID NO: 118 - protein, 10 aa, synthetic construct
  REGION 1..10: note = 10G11 General Formula CDR1 G
  SITE 1: note = misc_feature - X is K, R, H
  SITE 2: note = misc_feature - X is S, K, R, H
  SITE 3: note = misc_feature - X is I, K, R, H
  SITE 5: note = misc_feature - X is S, K, R, H
XXXFXINAMD

SEQ ID NO: 119 - protein, 10 aa, synthetic construct
  REGION 1..10: note = 10G11 General Formula CDR1 H
  REGION 2..3: note = misc_feature - X is G, A, V, L, I, M, P, F, W, S, T, N, Q, Y, C, K, R, H, D, E
  SITE 5: note = misc_feature - X is G, A, V, L, I, M, P, F, W, S, T, N, Q, Y, C, K, R, H, D, E
RXXFXINAMD

SEQ ID NO: 120 - protein, 10 aa, synthetic construct
  REGION 1..10: note = 10G11 General Formula CDR1 I
  REGION 2..3: note = misc_feature - X is G, A, V, L, I, M, P, F, W, S, T, N, Q, Y, C, K, R, H
  SITE 5: note = misc_feature - X is G, A, V, L, I, M, P, F, W, S, T, N, Q, Y, C, K, R, H
RXXFXINAMD

SEQ ID NO: 121 - protein, 10 aa, synthetic construct
  REGION 1..10: note = 10G11 General Formula CDR1 J
  SITE 2: note = misc_feature - X is S, T, C, P, N, Q, K, R, H
  SITE 3: note = misc_feature - X is I, G, A, V, M, L, K, R, H
  SITE 5: note = misc_feature - X is S, T, C, P, N, Q, K, R, H
RXXFXINAMD

SEQ ID NO: 122 - protein, 10 aa, synthetic construct
  REGION 1..10: note = 10G11 General Formula CDR1 K
  SITE 2: note = misc_feature - X is S, K, R, H
  SITE 3: note = misc_feature - X is I, K, R, H
  SITE 5: note = misc_feature - X is S, K, R, H
RXXFXINAMD

SEQ ID NO: 123 - protein, 9 aa, synthetic construct
  REGION 1..9: note = 10G11 General Formula CDR2 A
  SITE 4: note = misc_feature - X is G, A, V, L, I, M, P, F, W, S, T, N, Q, Y, C, K, R, H, D, E
  SITE 9: note = misc_feature - X is G, A, V, L, I, M, P, F, W, S, T, N, Q, Y, C, K, R, H, D, E
GITXGGTTX

SEQ ID NO: 124 - protein, 9 aa, synthetic construct
  REGION 1..9: note = 10G11 General Formula CDR2 B
  SITE 4: note = misc_feature - X is any naturally occurring amino acid, except E or D
  SITE 9: note = misc_feature - X is G, A, V, L, I, M, P, F, W, S, T, N, Q, Y, C, K, R, H
GITXGGTTX

SEQ ID NO: 125 - protein, 9 aa, synthetic construct
  REGION 1..9: note = 10G11 General Formula CDR2 C
  SITE 4: note = misc_feature - X is G, A, V, M, L, I, K, R, H
  SITE 9: note = misc_feature - X is G, A, V, M, L, I, K, R, H
GITXGGTTX

SEQ ID NO: 126 - protein, 9 aa, synthetic construct
  REGION 1..9: note = 10G11 General Formula CDR2 D
  SITE 4: note = misc_feature - X is A, K, R, H
  SITE 9: note = misc_feature - X is A, K, R, H
GITXGGTTX

SEQ ID NO: 127 - protein, 9 aa, synthetic construct
  REGION 1..9: note = 10G11 General Formula CDR2 E
  SITE 4: note = misc_feature - X is A, K, R, H
  SITE 9: note = misc_feature - X is A, K, R, H
GITXGGTTX

SEQ ID NO: 128 - protein, 9 aa, synthetic construct
  REGION 1..9: note = 10G11 General Formula CDR2 F
  SITE 4: note = misc_feature - X is A, K, R, H
  SITE 9: note = misc_feature - X is A, K, R, H
GITXGGTTX

SEQ ID NO: 129 - protein, 9 aa, synthetic construct
  REGION 1..9: note = 10G11 General Formula CDR2 G
  SITE 4: note = misc_feature - X is K, R, H
  SITE 9: note = misc_feature - X is K, R, H
GITXGGTTX

SEQ ID NO: 130 - protein, 9 aa, synthetic construct
  REGION 1..9: note = 10G11 General Formula CDR2 H
GITRGGTTK

SEQ ID NO: 131 - protein, 9 aa, synthetic construct
  REGION 1..9: note = 10G11 General Formula CDR2 I
GITRGGTTK

SEQ ID NO: 132 - protein, 9 aa, synthetic construct
  REGION 1..9: note = 10G11 General Formula CDR2 J
GITRGGTTK

SEQ ID NO: 133 - protein, 9 aa, synthetic construct
  REGION 1..9: note = 10G11 General Formula CDR2 K
GITRGGTTK

SEQ ID NO: 134 - protein, 11 aa, synthetic construct
  REGION 1..11: note = 10G11 General Formula CDR3 A
  SITE 2: note = misc_feature - X is G, A, V, L, I, M, P, F, W, S, T, N, Q, Y, C, K, R, H, D, E
  REGION 7..9: note = misc_feature - X is G, A, V, L, I, M, P, F, W, S, T, N, Q, Y, C, K, R, H, D, E
LXGEQPXXXDY

SEQ ID NO: 135 - protein, 11 aa, synthetic construct
  REGION 1..11: note = 10G11 General Formula CDR3 B
  SITE 2: note = misc_feature - X is X is G, A, V, L, I, M, P, F, W, S, T, N, Q, Y, C, K, R, H
  REGION 7..9: note = misc_feature - X is X is G, A, V, L, I, M, P, F, W, S, T, N, Q, Y, C, K, R, H
LXGEQPXXXDY

SEQ ID NO: 136 - protein, 11 aa, synthetic construct
  REGION 1..11: note = 10G11 General Formula CDR3 C
  SITE 2: note = misc_feature - X is G, A, V, M, L, I, K, R, H
  REGION 7..8: note = misc_feature - X is G, A, V, L, I, M, P, F, W, S, T, N, Q, Y, C, K, R, H
  SITE 9: note = misc_feature - X is G, A, V, M, L, I, K, R, H
LXGEQPXXXDY

SEQ ID NO: 137 - protein, 11 aa, synthetic construct
  REGION 1..11: note = 10G11 General Formula CDR3 D
  SITE 2: note = misc_feature - X is A, K, R, H
  REGION 7..8: note = misc_feature - X is G, A, V, L, I, M, P, F, W, S, T, N, Q, Y, C, K, R, H
  SITE 9: note = misc_feature - X is A, K, R, H
LXGEQPXXXDY

SEQ ID NO: 138 - protein, 11 aa, synthetic construct
  REGION 1..11: note = 10G11 General Formula CDR3 E
  SITE 2: note = misc_feature - X is A, K, R, H
  SITE 7: note = misc_feature - X is W, F, Y, K, R, H
  SITE 8: note = misc_feature - X is S, T, C, P, N, Q, K, R, H
  SITE 9: note = misc_feature - X is A, K, R, H
LXGEQPXXXDY

SEQ ID NO: 139 - protein, 11 aa, synthetic construct
  REGION 1..11: note = 10G11 General Formula CDR3 F
  SITE 2: note = misc_feature - X is A, K, R, H
  SITE 7: note = misc_feature - X is W, K, R, H
  SITE 8: note = misc_feature - X is T, K, R, H
  SITE 9: note = misc_feature - X is A, K, R, H
LXGEQPXXXDY

SEQ ID NO: 140 - protein, 11 aa, synthetic construct
  REGION 1..11: note = 10G11 General Formula CDR3 G
  SITE 2: note = misc_feature - X is K, R, H
  SITE 7: note = misc_feature - X is W, K, R, H
  SITE 8: note = misc_feature - X is T, K, R, H
  SITE 9: note = misc_feature - X is K, R, H
LXGEQPXXXDY

SEQ ID NO: 141 - protein, 11 aa, synthetic construct
  REGION 1..11: note = 10G11 General Formula CDR3 H
  REGION 7..8: note = misc_feature - X is G, A, V, L, I, M, P, F, W, S, T, N, Q, Y, C, K, R, H, D, E
LRGEQPXXRDY

SEQ ID NO: 142 - protein, 11 aa, synthetic construct
  REGION 1..11: note = 10G11 General Formula CDR3 I
  REGION 7..8: note = misc_feature - X is G, A, V, L, I, M, P, F, W, S, T, N, Q, Y, C, K, R, H
LRGEQPXXRDY

SEQ ID NO: 143 - protein, 11 aa, synthetic construct
  REGION 1..11: note = 10G11 General Formula CDR3 J
  SITE 7: note = misc_feature - X is W, F, Y, K, R, H
  SITE 8: note = misc_feature - X is S, T, C, P, N, Q, K, R, H
LRGEQPXXRDY

SEQ ID NO: 144 - protein, 11 aa, synthetic construct
  REGION 1..11: note = 10G11 General Formula CDR3 K
  SITE 7: note = misc_feature - X is W, K, R, H
  SITE 8: note = misc_feature - X is T, K, R, H
LRGEQPXXRDY

SEQ ID NO: 145 - protein, 119 aa, synthetic construct
  REGION 1..119: note = Germline
  REGION 98..108: note = misc_feature - X is unknown
QVQLVESGGGLVQAGGSLRLSCAASGSIFSINAMGWYRQAPGKQRELVAAITSGGSTNYADSVKGRFTISRDNAKNTVYLQMNSLKPEDTAVYYCNAXXXXXXXXXXXWGQGTQVTVSS

SEQ ID NO: 146 - protein, 126 aa, synthetic construct
  REGION 1..126: note = 10E11Q-His
QVQLQESGGGLVQAGGSLRLSCAASGTIFRPTAMGWYRQAPGKERELVATITTGGSTKYADSVKGRFTISRGNAKNTVYLQMSSLKPEDTAVYYCNAQWGVRTRDYWGQGTQVTVSSAAAHHHHHH

SEQ ID NO: 147 - protein, 135 aa, synthetic construct
  REGION 1..135: note = 12C03Q-His
QVQLQESGGGLVQAGDSLRLSCAASISDRAFSRHVMGWFRQPPGKEREFVAAIGWTGRRTYYADSVKGRFTISRDNAMNTVYLQMNSLKPEDTAVYYCAASHFYSVSFEINDYDYWGQGTQVTVSSAAAHHHHHH

SEQ ID NO: 148 - protein, 128 aa, synthetic construct
  REGION 1..128: note = 10G11Q-His
QVQLQESGGGLVQAGGSLRLSCAASRSIFSINAMDWYRQAPGKQREWVAGITRGGTTKYADSVKGRFTISRDNAKKKVYLQMNSLKPEDTAVYYCNVLRGEQPWTRDYWGQGTQVTVSSAAAHHHHHH

SEQ ID NO: 149 - protein, 25 aa, synthetic construct
  REGION 1..25: note = 10G11 Framework region 1 (Q)
QVQLVESGGGLVQAGGSLRLSCAAS

SEQ ID NO: 150 - protein, 25 aa, synthetic construct
  REGION 1..25: note = 10G11 Framework region 1 (D)
DVQLVESGGGLVQAGGSLRLSCAAS

SEQ ID NO: 151 - protein, 14 aa, synthetic construct
  REGION 1..14: note = 10G11 Framework region 2
WYRQAPGKQREWVA

SEQ ID NO: 152 - protein, 39 aa, synthetic construct
  REGION 1..39: note = 10G11 Framework region 3
YADSVKGRFTISRDNAKKKVYLQMNSLKPEDTAVYYCNV

SEQ ID NO: 153 - protein, 11 aa, synthetic construct
  REGION 1..11: note = 10G11 and 10E11 Framework region 4
WGQGTQVTVSS

SEQ ID NO: 154 - protein, 25 aa, synthetic construct
  REGION 1..25: note = 10E11? Framework region 1 (Q)
QVQLQESGGGLVQAGGSLRLSCAAS

SEQ ID NO: 155 - protein, 25 aa, synthetic construct
  REGION 1..25: note = 10E11? Framework region 1 (D)
DVQLQESGGGLVQAGGSLRLSCAAS

SEQ ID NO: 156 - protein, 14 aa, synthetic construct
  REGION 1..14: note = 10E11? Framework region 2
WYRQAPGKERELVA

SEQ ID NO: 157 - protein, 39 aa, synthetic construct
  REGION 1..39: note = 10E11? Framework region 3
YADSVKGRFTISRGNAKNTVYLQMSSLKPEDTAVYYCNA

SEQ ID NO: 158 - protein, 25 aa, synthetic construct
  REGION 1..25: note = 12C03 Framework region 1 (Q)
QVQLQESGGGLVQAGDSLRLSCAAS

SEQ ID NO: 159 - protein, 25 aa, synthetic construct
  REGION 1..25: note = 12C03 Framework region 1 (D)
DVQLQESGGGLVQAGDSLRLSCAAS

SEQ ID NO: 160 - protein, 16 aa, synthetic construct
  REGION 1..16: note = 12C03 Framework region 2
MGWFRQPPGKEREFVA

SEQ ID NO: 161 - protein, 39 aa, synthetic construct
  REGION 1..39: note = 12C03 Framework region 3
YADSVKGRFTISRDNAMNTVYLQMNSLKPEDTAVYYCAA